European Patent Application EP 4 556 021 A1, published May 21, 2025. Title: SARS-COV-2 VACCINE BOOSTER COMPOSITION. Applicant: 에스케이바이오사이언스 주식회사. Application EP 23 840 034.5, filed July 12, 2023. The sequence listing filed with the application follows.

SEQUENCE LISTING (36 sequences)

SEQ ID NO: 1 - protein, 467 aa, synthetic construct
  source 1..467: note = Component A
MGILPSPGMPALLSLVSLLSVLLMGCVAETGTRFPNITNLCPFGEVFNATRFASVYAWNRKRISNCVADYSVLYNSASFSTFKCYGVSPTKLNDLCFTNVYADSFVIRGDEVRQIAPGQTGKIADYNYKLPDDFTGCVIAWNSNNLDSKVGGNYNYLYRLFRKSNLKPFERDISTEIYQAGSTPCNGVEGFNCYFPLQSYGFQPTNGVGYQPYRVVVLSFELLHAPATVCGPKKSTGGSGGSGSGGSGGSGSEKAAKAEEAARKMEELFKKHKIVAVLRANSVEEAIEKAVAVFAGGVHLIEITFTVPDADTVIKALSVLKEKGAIIGAGTVTSVEQARKAVESGAEFIVSPHLDEEISQFAKEKGVFYMPGVMTPTELVKAMKLGHTILKLFPGEVVGPQFVKAMKGPFPNVKFVPTGGVNLDNVAEWFKAGVLAVGVGSALVKGTPDEVREKAKAFVEKIRGATE

SEQ ID NO: 2 - protein, 157 aa, synthetic construct
  source 1..157: note = Component B
MNQHSHKDHETVRIAVVRARWHAEIVDACVSAFEAAMRDIGGDRFAVDVFDVPGAYEIPLHARTLAETGRYGAVLGTAFVVNGGIYRHEFVASAVINGMMNVQLNTGVPVLSAVLTPHNYDKSKAHTLLFLALFAVKGMEAARACVEILAAREKIAA

SEQ ID NO: 3 - DNA, 1404 bp, synthetic construct
  source 1..1404: mol_type = other DNA; note = Component A
atgggaatcctgccaagccctggaatgccagccctgctgtccctggtgtctctgctgagcgtgctgctgatgggatgcgtggcagagaccggaacaaggttccctaacatcaccaacctgtgcccattcggcgaggtgtttaacgccacacgctttgcctccgtgtatgcctggaaccggaagagaatctctaattgcgtggccgactatagcgtgctgtacaatagcgcctccttctctacctttaagtgctatggcgtgtctcccaccaagctgaacgacctgtgcttcacaaacgtgtacgccgacagctttgtgatccggggcgatgaggtgagacagatcgcaccaggacagaccggcaagatcgcagactacaactataagctgcctgacgatttcacaggctgcgtgatcgcctggaatagcaacaatctggattccaaagtgggcggcaactacaattatctgtacaggctgttccgcaagagcaacctgaagccatttgagcgggacatcagcaccgagatctaccaggcaggctccacaccatgcaacggagtggagggcttcaattgttattttcccctgcagagctacggcttccagcctaccaatggcgtgggctatcagccatacagagtggtggtgctgtcctttgagctgctgcacgcaccagcaaccgtgtgcggacctaagaagtccacaggcggctctggaggaagcggatccggaggatccggaggatctggaagcgagaaggcagcaaaggcagaggaggcagcaaggaagatggaggagctgttcaagaagcacaagatcgtggccgtgctgagagccaactctgtggaggaggccatcgagaaggcagtggccgtgttcgcaggaggagtgcacctgatcgagatcacctttacagtgcccgacgccgataccgtgatcaaggccctgtccgtgctgaaggagaagggagcaatcatcggagcaggaaccgtgacatctgtggagcaggcaaggaaggcagtggagtccggagccgagtttatcgtgtctcctcacctggatgaggagatctcccagttcgccaaggagaagggcgtgttttacatgcctggcgtgatgaccccaacagagctggtgaaggccatgaagctgggccacaccatcctgaagctgttcccaggagaggtggtgggaccacagtttgtgaaggccatgaagggcccattccccaatgtgaagtttgtgcctacaggcggcgtgaacctggacaatgtggcagagtggttcaaggcaggcgtgctggcagtgggagtgggatctgccctggtgaagggaaccccagatgaggtgagggaaaaggccaaggcctttgtggagaagatcaggggagcaacagagtga

SEQ ID NO: 4 - DNA, 474 bp, synthetic construct
  source 1..474: mol_type = other DNA; note = Component B
atgaaccagcacagtcacaaggaccacgaaacggtaagaatagcggtagtgcgtgcgcgttggcatgcggaaattgtggacgcctgtgtgagtgcgtttgaagccgcgatgcgtgatattggcggcgatcgttttgccgtggatgtgtttgatgtgccgggtgcgtacgaaattccactgcatgcgcgtaccctggcggaaaccggccgttatggcgcggtgttaggcaccgcctttgtggtgaatggtggcatttatcgtcacgaatttgtggcgagcgcggttattaacggcatgatgaatgtgcagctgaacacgggcgtgccagtgttaagtgccgtgctgaccccacacaactatgataaaagcaaagcccataccctgctgttcttagcgctgtttgcggtgaaaggcatggaagcggcgcgtgcctgcgtggagattttagcggcccgtgaaaagattgcggcgtga

SEQ ID NO: 5 - protein, 205 aa, synthetic construct
  source 1..205: note = I53-50A
MKMEELFKKHKIVAVLRANSVEEAIEKAVAVFAGGVHLIEITFTVPDADTVIKALSVLKEKGAIIGAGTVTSVEQARKAVESGAEFIVSPHLDEEISQFAKEKGVFYMPGVMTPTELVKAMKLGHTILKLFPGEVVGPQFVKAMKGPFPNVKFVPTGGVNLDNVAEWFKAGVLAVGVGSALVKGTPDEVREKAKAFVEKIRGATE

SEQ ID NO: 6 - protein, 205 aa, synthetic construct
  REGION 1..205: note = synthetically constructed nanostructure polypeptide
MKMEELFKKHKIVAVLRANSVEEAIEKAVAVFAGGVHLIEITFTVPDADTVIKALSVLKEKGAIIGAGTVTSVEQCRKAVESGAEFIVSPHLDEEISQFCKEKGVFYMPGVMTPTELVKAMKLGHTILKLFPGEVVGPQFVKAMKGPFPNVKFVPTGGVNLDNVCEWFKAGVLAVGVGSALVKGTPDEVREKAKAFVEKIRGCTE

SEQ ID NO: 7 - protein, 205 aa, synthetic construct
  REGION 1..205: note = synthetically constructed nanostructure polypeptide
MKMEELFKKHKIVAVLRANSVEEAIEKAVAVFAGGVHLIEITFTVPDADTVIKALSVLKEKGAIIGAGTVTSVEQCRKAVESGAEFIVSPHLDEEISQFCKEKGVFYMPGVMTPTELVKAMKLGHDILKLFPGEVVGPQFVKAMKGPFPNVKFVPTGGVNLDNVCEWFKAGVLAVGVGDALVKGDPDEVREKAKKFVEKIRGCTE

SEQ ID NO: 8 - protein, 205 aa, synthetic construct
  REGION 1..205: note = synthetically constructed nanostructure polypeptide
MKMEELFKKHKIVAVLRANSVEEAIEKAVAVFAGGVHLIEITFTVPDADTVIKALSVLKEKGAIIGAGTVTSVEQCRKAVESGAEFIVSPHLDEEISQFCKEKGVFYMPGVMTPTELVKAMKLGHDILKLFPGEVVGPEFVEAMKGPFPNVKFVPTGGVDLDDVCEWFDAGVLAVGVGDALVEGDPDEVREDAKEFVEEIRGCTE

SEQ ID NO: 9 - protein, 205 aa, synthetic construct
  REGION 1..205: note = synthetically constructed nanostructure polypeptide
MKMEELFKKHKIVAVLRANSVEEAIEKAVAVFAGGVHLIEITFTVPDADTVIKALSVLKEKGAIIGAGTVTSVEQCRKAVESGAEFIVSPHLDEEISQFCKEKGVFYMPGVMTPTELVKAMKLGHDILKLFPGEVVGPQFVKAMKGPFPNVKFVPTGGVNLDNVCKWFKAGVLAVGVGKALVKGKPDEVREKAKKFVKKIRGCTE

SEQ ID NO: 10 - protein, 205 aa, synthetic construct
  REGION 1..205: note = synthetically constructed nanostructure polypeptide
  SITE 126: note = MISC_FEATURE - Xaa is Thr or Asp
  SITE 139: note = MISC_FEATURE - Xaa is Gln or Glu
  SITE 142: note = MISC_FEATURE - Xaa is Lys or Glu
  SITE 160: note = MISC_FEATURE - Xaa is Asn or Asp
  SITE 163: note = MISC_FEATURE - Xaa is Asn or Asp
  SITE 166: note = MISC_FEATURE - Xaa is Glu or Lys
  SITE 169: note = MISC_FEATURE - Xaa is Lys or Asp
  SITE 179: note = MISC_FEATURE - Xaa is Ser, Lys or Asp
  SITE 183: note = MISC_FEATURE - Xaa is Lys or Glu
  SITE 185: note = MISC_FEATURE - Xaa is Thr, Asp or Lys
  SITE 192: note = MISC_FEATURE - Xaa is Lys or Asp
  SITE 195: note = MISC_FEATURE - Xaa is Ala, Glu or Lys
  SITE 198: note = MISC_FEATURE - Xaa is Glu or Lys
  SITE 199: note = MISC_FEATURE - Xaa is Lys or Glu
MKMEELFKKHKIVAVLRANSVEEAIEKAVAVFAGGVHLIEITFTVPDADTVIKALSVLKEKGAIIGAGTVTSVEQCRKAVESGAEFIVSPHLDEEISQFCKEKGVFYMPGVMTPTELVKAMKLGHXILKLFPGEVVGPXFVXAMKGPFPNVKFVPTGGVXLDXVCXWFXAGVLAVGVGXALVXGXPDEVREXAKXFVXXIRGCTE

SEQ ID NO: 11 - protein, 157 aa, synthetic construct
  REGION 1..157: note = synthetically constructed nanostructure polypeptide
MNQHSHKDYETVRIAVVRARWHADIVDACVEAFEIAMAAIGGDRFAVDVFDVPGAYEIPLHARTLAETGRYGAVLGTAFVVNGGIYRHEFVASAVIDGMMNVQLSTGVPVLSAVLTPHRYRDSAEHHRFFAAHFAVKGVEAARACIEILAAREKIAA

SEQ ID NO: 12 - protein, 157 aa, synthetic construct
  REGION 1..157: note = synthetically constructed nanostructure polypeptide
MNQHSHKDYETVRIAVVRARWHAEIVDACVSAFEAAMADIGGDRFAVDVFDVPGAYEIPLHARTLAETGRYGAVLGTAFVVNGGIYRHEFVASAVIDGMMNVQLSTGVPVLSAVLTPHRYRDSDAHTLLFLALFAVKGMEAARACVEILAAREKIAA

SEQ ID NO: 13 - protein, 157 aa, synthetic construct
  REGION 1..157: note = synthetically constructed nanostructure polypeptide
MNQHSHKDYETVRIAVVRARWHADIVDQCVRAFEEAMADAGGDRFAVDVFDVPGAYEIPLHARTLAETGRYGAVLGTAFVVNGGIYRHEFVASAVIDGMMNVQLSTGVPVLSAVLTPHRYRSSREHHEFFREHFMVKGVEAAAACITILAAREKIAA

SEQ ID NO: 14 - protein, 157 aa, synthetic construct
  REGION 1..157: note = synthetically constructed nanostructure polypeptide
MNQHSHKDHETVRIAVVRARWHADIVDACVEAFEIAMAAIGGDRFAVDVFDVPGAYEIPLHARTLAETGRYGAVLGTAFVVNGGIYRHEFVASAVIDGMMNVQLDTGVPVLSAVLTPHRYRDSDEHHRFFAAHFAVKGVEAARACIEILNAREKIAA

SEQ ID NO: 15 - protein, 157 aa, synthetic construct
  REGION 1..157: note = synthetically constructed nanostructure polypeptide
MNQHSHKDHETVRIAVVRARWHADIVDACVEAFEIAMAAIGGDRFAVDVFDVPGAYEIPLHARTLAETGRYGAVLGTAFVVDGGIYDHEFVASAVIDGMMNVQLDTGVPVLSAVLTPHEYEDSDEDHEFFAAHFAVKGVEAARACIEILNAREKIAA

SEQ ID NO: 16 - protein, 157 aa, synthetic construct
  REGION 1..157: note = synthetically constructed nanostructure polypeptide
MNQHSHKDHETVRIAVVRARWHAEIVDACVSAFEAAMRDIGGDRFAVDVFDVPGAYEIPLHARTLAETGRYGAVLGTAFVVNGGIYRHEFVASAVIDGMMNVQLDTGVPVLSAVLTPHRYRDSDAHTLLFLALFAVKGMEAARACVEILAAREKIAA

SEQ ID NO: 17 - protein, 157 aa, synthetic construct
  REGION 1..157: note = synthetically constructed nanostructure polypeptide
MNQHSHKDHETVRIAVVRARWHAEIVDACVSAFEAAMRDIGGDRFAVDVFDVPGAYEIPLHARTLAETGRYGAVLGTAFVVDGGIYDHEFVASAVIDGMMNVQLDTGVPVLSAVLTPHEYEDSDADTLLFLALFAVKGMEAARACVEILAAREKIAA

SEQ ID NO: 18 - protein, 157 aa, synthetic construct
  REGION 1..157: note = synthetically constructed nanostructure polypeptide
  SITE 9: note = MISC_FEATURE - Xaa is Tyr or His
  SITE 82: note = MISC_FEATURE - Xaa is Asn or Asp
  SITE 87: note = MISC_FEATURE - Xaa is Arg or Asp
  SITE 105: note = MISC_FEATURE - Xaa is Ser or Asp
  SITE 119: note = MISC_FEATURE - Xaa is Arg or Glu
  SITE 121: note = MISC_FEATURE - Xaa is Arg or Glu
  SITE 124: note = MISC_FEATURE - Xaa is Ala or Asp
  SITE 126: note = MISC_FEATURE - Xaa is His or Asp
  SITE 128: note = MISC_FEATURE - Xaa is Arg or Glu
  SITE 150: note = MISC_FEATURE - Xaa is Ala or Asn
MNQHSHKDXETVRIAVVRARWHADIVDACVEAFEIAMAAIGGDRFAVDVFDVPGAYEIPLHARTLAETGRYGAVLGTAFVVXGGIYXHEFVASAVIDGMMNVQLXTGVPVLSAVLTPHXYXDSXEXHXFFAAHFAVKGVEAARACIEILXAREKIAA

SEQ ID NO: 19 - DNA, 10704 bp, synthetic construct
  source 1..10704: mol_type = other DNA; note = plasmid ComA
tcgcgcgtttcggtgatgacggtgaaaacctctgacacatgcagctcccggagacggtcacagcttgtctgtaagcggatgccgggagcagacaagcccgtcagggcgcgtcagcgggtgttggcgggtgtcggggctggcttaactatgcggcatcagagcagattgtactgagagtgcaccatatgcggtgtgaaataccgcacagatgcgtaaggagaaaataccgcatcaggcgccattcgccattcaggctgcgcaactgttgggaagggcgatcggtgcgggcctcttcgctattacgccagctggcgaaagggggatgtgctgcaaggcgattaagttgggtaacgccagggttttcccagtcacgacgttgtaaaacgacggccagtgaattggagatcggtacttcgcgaatgcgtcgagatgtttaaactcccgcccctaactccgcccagttccgcccattctccgccccatggctgactaattttttttatttatgcagaggccgaggccgcctcggcctctgagctattccagaagtagtgaggaggcttttttggaggcctaggcttttgcaaaaagctagctggttctttccgcctcagaaggtacctaaccaagttcctctttcagaggttatttcaggccaccttccaccatggccacctcagcaagttcccacttgaacaaaaacatcaagcaaatgtacttgtgcctgccccagggtgagaaagtccaagccatgtatatctgggttgatggtactggagaaggactgcgctgcaaaacccgcaccctggactgtgagcccaagtgtgtagaagagttacctgagtggaattttgatggctctagtacctttcagtctgagggctccaacagtgacatgtatctcagccctgttgccatgtttcgggaccccttccgcagagatcccaacaagctggtgttctgtgaagttttcaagtacaaccggaagcctgcagagaccaatttaaggcactcgtgtaaacggataatggacatggtgagcaaccagcacccctggtttggaatggaacaggagtatactctgatgggaacagatgggcacccttttggttggccttccaatggctttcctgggccccaaggtccgtattactgtggtgtgggcgcagacaaagcctatggcagggatatcgtggaggctcactaccgcgcctgcttgtatgctggggtcaagattacaggaacaaatgctgaggtcatgcctgcccagtgggaatttcaaataggaccctgtgaaggaatccgcatgggagatcatctctgggtggcccgtttcatcttgcatcgagtatgtgaagactttggggtaatagcaacctttgaccccaagcccattcctgggaactggaatggtgcaggctgccataccaactttagcaccaaggccatgcgggaggagaatggtctgaagcacatcgaggaggccatcgagaaactaagcaagcggcaccggtaccacattcgagcctacgatcccaaggggggcctggacaatgcccgtcgtctgactgggttccacgaaacgtccaacatcaacgacttttctgctggtgtcgccaatcgcagtgccagcatccgcattccccggactgtcggccaggagaagaaaggttactttgaagaccgccgcccctctgccaattgtgacccctttgcagtgacagaagccatcgtccgcacatgccttctcaatgagactggcgacgagcccttccaatacaaaaactaacgcccgccccacgacccgcagcgcccgaccgaaaggagcgcacgaccccatgcatcgcacacatcataagatacattgatgagtttggacaaaccacaactagaatgcagtgaaaaaaatgctttatttgtgaaatttgtgatgctattgctttatttgtaaccattataagctgcaataaacaagttaacaacaacaattgcattcattttatgtttcaggttcagggggagatgtgggaggttttttaaagcaagtaaaacctctacaaatgtggtagaattctacgtagataaaagttttgttactttatagaagaaattttgagtttttgttttttttaataaataaataaacataaataaattgtttgttgaatttattattagtatgtaagtgtaaatataataaaacttaatatctattcaaattaataaataaacctcgatatacagaccgataaaacacatgcgtcaattttacacatgattatctttaacgtacgtcacaatatgattatctttctagggttaatctagctgcgtgttctgcagcgtgtcgagcatcttcatctgctccatcacgctgtaaaacacatttgcaccgcgagtctgcccgtcctccacgggttcaaaaacgtgaatgaacgaggcgcgctcatatcatgattacgccaagcgcgcccgccgggtaactcacggggtatccatgtccatttctgcggcatccagccaggatacccgtcctcgctgacgtaatatcccagcgccgcaccgctgtcattaatctgcacaccggcacggcagttccatttaaatggctgtcgccggtattgttcgggttgctgatgcgcttcgggctgaccatccggaactgtgtccggaaaagccgcgacgaactggtatcccaggtggcctgaacgaacagttcaccgttaaaggcgtgcatggccacaccttcccgaatcatcatggtaaacgtgcgttttcgctcaacgtcaatgcagcagcagtcatcctcggcaaactctttccatgccgcttcaacctcgcgggaaaaggcacgggcttcttcctccccgatgcccagatagcgccagcttgggcgatgactgagccggaaaaaagacccgacgatatgatcctgatgcagctagattaaccctagaaagatagtctgcgtaaaattgacgcatgcattcttgaaatattgctctctctttctaaatagcgcgaatccgtcgctgtgcatttaggacatctcagtcgccgcttggagctcccgtgaggcgtgcttgtcaatgcggtaagtgtcactgattttgaactataacgaccgcgtgagtcaaaatgacgcatgattatcttttacgtgacttttaagatttaactcatacgataattatattgttatttcatgttctacttacgtgataacttattatatatatattttcttgttatagatatcaagcttatagatctggggacagcccccccccaaagcccccagggatgtaattacgtccctcccccgctagggggcagcagcgagccgcccggggctccgctccggtccggcgctccccccgcatccccgagccggcagcgtgcggggacagcccgggcacggggaaggtggcacgggatcgctttcctctgaacgcttctcgctgctctttgagcctgcagacacctggggggatacggggaaaaagctttaggctgaaagagagatttagaatgacagaatcatagaacggcctgggttgcaaaggagcacagtgctcatccagatccaaccccctgctatgtgcagggtcatcaaccagcagcccaggctgcccagagccacatccagcctggccttgaatgcctgcagggatggggcatccacagcctccttgggcaacctgttcagtgcgtcaccaccctctgggggaaaaactgcctcctcatatccaacccaaacctcccctgtctcagtgtaaagccattcccccttgtcctatcaagggggagtttgctgtgacattgttggtctggggtgacacatgtttgccaattcagtgcatcacggagaggcagatttggggataaggaagtgcaggacagcatggacgtgggacatgcaggtgttgagggctctgggacactctccaagtcacagcgttcagaacagccttaaggataagaagataggatagaaggacaaagagcaagttaaaacccagcatggagaggagcacaaaaaggccacagacactgctggtccctgtgtctgagcctgcatgtttgatggtgtctggatgcaagcagaaggggtggaagagcttgcctggagagatacagctgggtcagtaggactgggacaggcagctggagaattgccatgtagatgttcatacaatcgtcaaatcatgaaggctggaaaagccctccaagatccccaagaccaaccccaacccacccaccgtgcccactggccatgtccctcagtgccacatccccacagttcttcatcacctccagggacggtgacccccccacctccgtgggcagctgtgccactgcagcaccgctctttggagaaggtaaatcttgctaaatccagcccgaccctcccctggcacaacgtaaggccattatctctcatccaactccaggacggagtcagtgaggatggggctctagagtcaacaggaaagttccattggagccaagtacattgagtcaatagggactttccaatgggttttgcccagtacataaggtcaatgggaggtaagccaatgggtttttcccattactggcacgtatactgagtcattagggactttccaatgggttttgcccagtacataaggtcaataggggtgaatcaacaggaaagtcccattggagccaagtacactgagtcaatagggactttccattgggttttgcccagtacaaaaggtcaatagggggtgagtcaatgggtttttcccattattggcacgtacataaggtcaataggggtgagtcattgggtttttccagccaatttaattaaaacgccatgtactttcccaccattgacgtcaatgggctattgaaactaatgcaacgtgacctttaaacggtactttcccatagctgattaatgggaaagtaccgttctcgagccaatacacgtcaatgggaagtgaaagggcagccaaaacgtaacaccgccccggttttcccctggaaattccatattggcacgcattctattggctgagctgcgttctacgtgggtatataagcagagctctccctatcagtgatagagatctccctatcagtgatagagatcgagctcagcgtcggtaccgtacctcttccgcatcgctgtctgcgagggccagctgttggggtgagtggcgggtgtggcttccgcgggccccggagctggagccctgctctgagcgggccgggctgatatgcgagtgtcgtccgcagggtttagctgtgagcattcccacttcgagtggcgggcggtgcgggggtgagagtgcgaggcctagcggcaaccccgtagcctcgcctcgtgtccggcttgaggcctagcgtggtgtccgccgccgcgtgccactccggccgcactatgcgttttttgtccttgctgccctcgattgccttccagcagcatgggctaacaaagggagggtgtggggctcactcttaaggagcccatgaagcttacgttggataggaatggaagggcaggaggggcgactggggcccgcccgccttcggagcacatgtccgacgccacctggatggggcgaggcctgtggctttccgaagcaatcgggcgtgagtttagcctacctgggccatgtggccctagcactgggcacggtctggcctggcggtgccgcgttcccttgcctcccaacaagggtgaggccgtcccgcccggcaccagttgcttgcgcggaaagatggccgctcccggggccctgttgcaaggagctcaaaatggaggacgcggcagcccggtggagcgggcgggtgagtcacccacacaaaggaagagggccttgcccctcgccggccgctgcttcctgtgaccccgtggtctatcggccgcatagtcacctcgggcttctcttgagcaccgctcgtcgcggcggggggaggggatctaatggcgttggagtttgttcacatttggtgggtggagactagtcaggccagcctggcgctggaagtcattcttggaatttgcccctttgagtttggagcgaggctaattctcaagcctcttagcggttcaaaggtattttctaaacccgtttccagctcgcggttgaggacaaactcttcgcggtctttccagtactcttggatcggaaacccgtcggcctccgaacggtactccgccaccgagggacctgagcgagtccgcatcgaccggatcggaaaacctcgtcgacgccgccaccatgggaatcctgccaagccctggaatgccagccctgctgtccctggtgtctctgctgagcgtgctgctgatgggatgcgtggcagagaccggaacaaggttccctaacatcaccaacctgtgcccattcggcgaggtgtttaacgccacacgctttgcctccgtgtatgcctggaaccggaagagaatctctaattgcgtggccgactatagcgtgctgtacaatagcgcctccttctctacctttaagtgctatggcgtgtctcccaccaagctgaacgacctgtgcttcacaaacgtgtacgccgacagctttgtgatccggggcgatgaggtgagacagatcgcaccaggacagaccggcaagatcgcagactacaactataagctgcctgacgatttcacaggctgcgtgatcgcctggaatagcaacaatctggattccaaagtgggcggcaactacaattatctgtacaggctgttccgcaagagcaacctgaagccatttgagcgggacatcagcaccgagatctaccaggcaggctccacaccatgcaacggagtggagggcttcaattgttattttcccctgcagagctacggcttccagcctaccaatggcgtgggctatcagccatacagagtggtggtgctgtcctttgagctgctgcacgcaccagcaaccgtgtgcggacctaagaagtccacaggcggctctggaggaagcggatccggaggatccggaggatctggaagcgagaaggcagcaaaggcagaggaggcagcaaggaagatggaggagctgttcaagaagcacaagatcgtggccgtgctgagagccaactctgtggaggaggccatcgagaaggcagtggccgtgttcgcaggaggagtgcacctgatcgagatcacctttacagtgcccgacgccgataccgtgatcaaggccctgtccgtgctgaaggagaagggagcaatcatcggagcaggaaccgtgacatctgtggagcaggcaaggaaggcagtggagtccggagccgagtttatcgtgtctcctcacctggatgaggagatctcccagttcgccaaggagaagggcgtgttttacatgcctggcgtgatgaccccaacagagctggtgaaggccatgaagctgggccacaccatcctgaagctgttcccaggagaggtggtgggaccacagtttgtgaaggccatgaagggcccattccccaatgtgaagtttgtgcctacaggcggcgtgaacctggacaatgtggcagagtggttcaaggcaggcgtgctggcagtgggagtgggatctgccctggtgaagggaaccccagatgaggtgagggaaaaggccaaggcctttgtggagaagatcaggggagcaacagagtgagcggccgccacacatcataagatacattgatgagtttggacaaaccacaactagaatgcagtgaaaaaaatgctttatttgtgaaatttgtgatgctattgctttatttgtaaccattataagctgcaataaacaagttaacaacaacaattgcattcattttatgtttcaggttcagggggagatgtgggaggttttttaaagcaagtaaaacctctacaaatgtggtacacaaagtggggagctctagagggacagcccccccccaaagcccccagggatgtaattacgtccctcccccgctagggggcagcagcgagccgcccggggctccgctccggtccggcgctccccccgcatccccgagccggcagcgtgcggggacagcccgggcacggggaaggtggcacgggatcgctttcctctgaacgcttctcgctgctctttgagcctgcagacacctggggggatacggggaaaaaggggagctctagagggacagcccccccccaaagcccccagggatgtaattacgtccctcccccgctagggggcagcagcgagccgcccggggctccgctccggtccggcgctccccccgcatccccgagccggcagcgtgcggggacagcccgggcacggggaaggtggcacgggatcgctttcctctgaacgcttctcgctgctctttgagcctgcagacacctggggggatacggggaaaaaggatccatggccggccatctgcagatcatatgatcggatgccgggaccgacgagtgcagaggcgtgcaagcgagcttggcgtaatcatggtcatagctgtttcctgtgtgaaattgttatccgctcacaattccacacaacatacgagccggaagcataaagtgtaaagcctggggtgcctaatgagtgagctaactcacattaattgcgttgcgctcactgcccgctttccagtcgggaaacctgtcgtgccagctgcattaatgaatcggccaacgcgcggggagaggcggtttgcgtattgggcgctcttccgcttcctcgctcactgactcgctgcgctcggtcgttcggctgcggcgagcggtatcagctcactcaaaggcggtaatacggttatccacagaatcaggggataacgcaggaaagaacatgtgagcaaaaggccagcaaaaggccaggaaccgtaaaaaggccgcgttgctggcgtttttccataggctccgcccccctgacgagcatcacaaaaatcgacgctcaagtcagaggtggcgaaacccgacaggactataaagataccaggcgtttccccctggaagctccctcgtgcgctctcctgttccgaccctgccgcttaccggatacctgtccgcctttctcccttcgggaagcgtggcgctttctcatagctcacgctgtaggtatctcagttcggtgtaggtcgttcgctccaagctgggctgtgtgcacgaaccccccgttcagcccgaccgctgcgccttatccggtaactatcgtcttgagtccaacccggtaagacacgacttatcgccactggcagcagccactggtaacaggattagcagagcgaggtatgtaggcggtgctacagagttcttgaagtggtggcctaactacggctacactagaagaacagtatttggtatctgcgctctgctgaagccagttaccttcggaaaaagagttggtagctcttgatccggcaaacaaaccaccgctggtagcggtggtttttttgtttgcaagcagcagattacgcgcagaaaaaaaggatctcaagaagatcctttgatcttttctacggggtctgacgctcagtggaacgaaaactcacgttaagggattttggtcatgagattatcaaaaaggatcttcacctagatccttttaaattaaaaatgaagttttaaatcaatctaaagtatatatgagtaaacttggtctgacagttaccaatgcttaatcagtgaggcacctatctcagcgatctgtctatttcgttcatccatagttgcctgactccccgtcgtgtagataactacgatacgggagggcttaccatctggccccagtgctgcaatgataccgcgagacccacgctcaccggctccagatttatcagcaataaaccagccagccggaagggccgagcgcagaagtggtcctgcaactttatccgcctccatccagtctattaattgttgccgggaagctagagtaagtagttcgccagttaatagtttgcgcaacgttgttgccattgctacaggcatcgtggtgtcacgctcgtcgtttggtatggcttcattcagctccggttcccaacgatcaaggcgagttacatgatcccccatgttgtgcaaaaaagcggttagctccttcggtcctccgatcgttgtcagaagtaagttggccgcagtgttatcactcatggttatggcagcactgcataattctcttactgtcatgccatccgtaagatgcttttctgtgactggtgagtactcaaccaagtcattctgagaatagtgtatgcggcgaccgagttgctcttgcccggcgtcaatacgggataataccgcgccacatagcagaactttaaaagtgctcatcattggaaaacgttcttcggggcgaaaactctcaaggatcttaccgctgttgagatccagttcgatgtaacccactcgtgcacccaactgatcttcagcatcttttactttcaccagcgtttctgggtgagcaaaaacaggaaggcaaaatgccgcaaaaaagggaataagggcgacacggaaatgttgaatactcatactcttcctttttcaatattattgaagcatttatcagggttattgtctcatgagcggatacatatttgaatgtatttagaaaaataaacaaataggggttccgcgcacatttccccgaaaagtgccacctgacgtctaagaaaccattattatcatgacattaacctataaaaataggcgtatcacgaggccctttcgtc

SEQ ID NO: 20 - DNA, 5712 bp, synthetic construct
  source 1..5712: mol_type = other DNA; note = plasmid ComB
tggcgaatgggacgcgccctgtagcggcgcattaagcgcggcgggtgtggtggttacgcgcagcgtgaccgctacacttgccagcgccctagcgcccgctcctttcgctttcttcccttcctttctcgccacgttcgccggctttccccgtcaagctctaaatcgggggctccctttagggttccgatttagtgctttacggcacctcgaccccaaaaaacttgattagggtgatggttcacgtagtgggccatcgccctgatagacggtttttcgccctttgacgttggagtccacgttctttaatagtggactcttgttccaaactggaacaacactcaaccctatctcggtctattcttttgatttataagggattttgccgatttcggcctattggttaaaaaatgagctgatttaacaaaaatttaacgcgaattttaacaaaatattaacgtttacaatttcaggtggcacttttcggggaaatgtgcgcggaacccctatttgtttatttttctaaatacattcaaatatgtatccgctcatgaattaattcttagaaaaactcatcgagcatcaaatgaaactgcaatttattcatatcaggattatcaataccatatttttgaaaaagccgtttctgtaatgaaggagaaaactcaccgaggcagttccataggatggcaagatcctggtatcggtctgcgattccgactcgtccaacatcaatacaacctattaatttcccctcgtcaaaaataaggttatcaagtgagaaatcaccatgagtgacgactgaatccggtgagaatggcaaaagtttatgcatttctttccagacttgttcaacaggccagccattacgctcgtcatcaaaatcactcgcatcaaccaaaccgttattcattcgtgattgcgcctgagcgagacgaaatacgcgatcgctgttaaaaggacaattacaaacaggaatcgaatgcaaccggcgcaggaacactgccagcgcatcaacaatattttcacctgaatcaggatattcttctaatacctggaatgctgttttcccggggatcgcagtggtgagtaaccatgcatcatcaggagtacggataaaatgcttgatggtcggaagaggcataaattccgtcagccagtttagtctgaccatctcatctgtaacatcattggcaacgctacctttgccatgtttcagaaacaactctggcgcatcgggcttcccatacaatcgatagattgtcgcacctgattgcccgacattatcgcgagcccatttatacccatataaatcagcatccatgttggaatttaatcgcggcctagagcaagacgtttcccgttgaatatggctcataacaccccttgtattactgtttatgtaagcagacagttttattgttcatgaccaaaatcccttaacgtgagttttcgttccactgagcgtcagaccccgtagaaaagatcaaaggatcttcttgagatcctttttttctgcgcgtaatctgctgcttgcaaacaaaaaaaccaccgctaccagcggtggtttgtttgccggatcaagagctaccaactctttttccgaaggtaactggcttcagcagagcgcagataccaaatactgtccttctagtgtagccgtagttaggccaccacttcaagaactctgtagcaccgcctacatacctcgctctgctaatcctgttaccagtggctgctgccagtggcgataagtcgtgtcttaccgggttggactcaagacgatagttaccggataaggcgcagcggtcgggctgaacggggggttcgtgcacacagcccagcttggagcgaacgacctacaccgaactgagatacctacagcgtgagctatgagaaagcgccacgcttcccgaagggagaaaggcggacaggtatccggtaagcggcagggtcggaacaggagagcgcacgagggagcttccagggggaaacgcctggtatctttatagtcctgtcgggtttcgccacctctgacttgagcgtcgatttttgtgatgctcgtcaggggggcggagcctatggaaaaacgccagcaacgcggcctttttacggttcctggccttttgctggccttttgctcacatgttctttcctgcgttatcccctgattctgtggataaccgtattaccgcctttgagtgagctgataccgctcgccgcagccgaacgaccgagcgcagcgagtcagtgagcgaggaagcggaagagcgcctgatgcggtattttctccttacgcatctgtgcggtatttcacaccgcatatatggtgcactctcagtacaatctgctctgatgccgcatagttaagccagtatacactccgctatcgctacgtgactgggtcatggctgcgccccgacacccgccaacacccgctgacgcgccctgacgggcttgtctgctcccggcatccgcttacagacaagctgtgaccgtctccgggagctgcatgtgtcagaggttttcaccgtcatcaccgaaacgcgcgaggcagctgcggtaaagctcatcagcgtggtcgtgaagcgattcacagatgtctgcctgttcatccgcgtccagctcgttgagtttctccagaagcgttaatgtctggcttctgataaagcgggccatgttaagggcggttttttcctgtttggtcactgatgcctccgtgtaagggggatttctgttcatgggggtaatgataccgatgaaacgagagaggatgctcacgatacgggttactgatgatgaacatgcccggttactggaacgttgtgagggtaaacaactggcggtatggatgcggcgggaccagagaaaaatcactcagggtcaatgccagcgcttcgttaatacagatgtaggtgttccacagggtagccagcagcatcctgcgatgcagatccggaacataatggtgcagggcgctgacttccgcgtttccagactttacgaaacacggaaaccgaagaccattcatgttgttgctcaggtcgcagacgttttgcagcagcagtcgcttcacgttcgctcgcgtatcggtgattcattctgctaaccagtaaggcaaccccgccagcctagccgggtcctcaacgacaggagcacgatcatgcgcacccgtggggccgccatgccggcgataatggcctgcttctcgccgaaacgtttggtggcgggaccagtgacgaaggcttgagcgagggcgtgcaagattccgaataccgcaagcgacaggccgatcatcgtcgcgctccagcgaaagcggtcctcgccgaaaatgacccagagcgctgccggcacctgtcctacgagttgcatgataaagaagacagtcataagtgcggcgacgatagtcatgccccgcgcccaccggaaggagctgactgggttgaaggctctcaagggcatcggtcgagatcccggtgcctaatgagtgagctaacttacattaattgcgttgcgctcactgcccgctttccagtcgggaaacctgtcgtgccagctgcattaatgaatcggccaacgcgcggggagaggcggtttgcgtattgggcgccagggtggtttttcttttcaccagtgagacgggcaacagctgattgcccttcaccgcctggccctgagagagttgcagcaagcggtccacgctggtttgccccagcaggcgaaaatcctgtttgatggtggttaacggcgggatataacatgagctgtcttcggtatcgtcgtatcccactaccgagatgtccgcaccaacgcgcagcccggactcggtaatggcgcgcattgcgcccagcgccatctgatcgttggcaaccagcatcgcagtgggaacgatgccctcattcagcatttgcatggtttgttgaaaaccggacatggcactccagtcgccttcccgttccgctatcggctgaatttgattgcgagtgagatatttatgccagccagccagacgcagacgcgccgagacagaacttaatgggcccgctaacagcgcgatttgctggtgacccaatgcgaccagatgctccacgcccagtcgcgtaccgtcttcatgggagaaaataatactgttgatgggtgtctggtcagagacatcaagaaataacgccggaacattagtgcaggcagcttccacagcaatggcatcctggtcatccagcggatagttaatgatcagcccactgacgcgttgcgcgagaagattgtgcaccgccgctttacaggcttcgacgccgcttcgttctaccatcgacaccaccacgctggcacccagttgatcggcgcgagatttaatcgccgcgacaatttgcgacggcgcgtgcagggccagactggaggtggcaacgccaatcagcaacgactgtttgcccgccagttgttgtgccacgcggttgggaatgtaattcagctccgccatcgccgcttccactttttcccgcgttttcgcagaaacgtggctggcctggttcaccacgcgggaaacggtctgataagagacaccggcatactctgcgacatcgtataacgttactggtttcacattcaccaccctgaattgactctcttccgggcgctatcatgccataccgcgaaaggttttgcgccattcgatggtgtccgggatctcgacgctctcccttatgcgactcctgcattaggaagcagcccagtagtaggttgaggccgttgagcaccgccgccgcaaggaatggtgcatgcaaggagatggcgcccaacagtcccccggccacggggcctgccaccatacccacgccgaaacaagcgctcatgagcccgaagtggcgagcccgatcttccccatcggtgatgtcggcgatataggcgccagcaaccgcacctgtggcgccggtgatgccggccacgatgcgtccggcgtagaggatcgagatcgatctcgatcccgcgaaattaatacgactcactataggggaattgtgagcggataacaattcccctctagaaataattttgtttaactttaagaaggagatatacatatgaaccagcacagtcacaaggaccacgaaacggtaagaatagcggtagtgcgtgcgcgttggcatgcggaaattgtggacgcctgtgtgagtgcgtttgaagccgcgatgcgtgatattggcggcgatcgttttgccgtggatgtgtttgatgtgccgggtgcgtacgaaattccactgcatgcgcgtaccctggcggaaaccggccgttatggcgcggtgttaggcaccgcctttgtggtgaatggtggcatttatcgtcacgaatttgtggcgagcgcggttattaacggcatgatgaatgtgcagctgaacacgggcgtgccagtgttaagtgccgtgctgaccccacacaactatgataaaagcaaagcccataccctgctgttcttagcgctgtttgcggtgaaaggcatggaagcggcgcgtgcctgcgtggagattttagcggcccgtgaaaagattgcggcgtgactcgagcaccaccaccaccaccactgagatccggctgctaacaaagcccgaaaggaagctgagttggctgctgccaccgctgagcaataactagcataaccccttggggcctctaaacgggtcttgaggggttttttgctgaaaggaggaactatatccggat

SEQ ID NO: 21 - protein, 204 aa, SARS-CoV-2 Wuhan-Hu-1
RFPNITNLCPFGEVFNATRFASVYAWNRKRISNCVADYSVLYNSASFSTFKCYGVSPTKLNDLCFTNVYADSFVIRGDEVRQIAPGQTGKIADYNYKLPDDFTGCVIAWNSNNLDSKVGGNYNYLYRLFRKSNLKPFERDISTEIYQAGSTPCNGVEGFNCYFPLQSYGFQPTNGVGYQPYRVVVLSFELLHAPATVCGPKKST

SEQ ID NO: 22 - protein, 204 aa, SARS-CoV-2 Beta
RFPNITNLCPFGEVFNATRFASVYAWNRKRISNCVADYSVLYNSASFSTFKCYGVSPTKLNDLCFTNVYADSFVIRGDEVRQIAPGQTGNIADYNYKLPDDFTGCVIAWNSNNLDSKVGGNYNYLYRLFRKSNLKPFERDISTEIYQAGSTPCNGVKGFNCYFPLQSYGFQPTYGVGYQPYRVVVLSFELLHAPATVCGPKKST

SEQ ID NO: 23 - protein, 204 aa, SARS-CoV-2 Delta
RFPNITNLCPFGEVFNATRFASVYAWNRKRISNCVADYSVLYNSASFSTFKCYGVSPTKLNDLCFTNVYADSFVIRGDEVRQIAPGQTGKIADYNYKLPDDFTGCVIAWNSNNLDSKVGGNYNYRYRLFRKSNLKPFERDISTEIYQAGSKPCNGVEGFNCYFPLQSYGFQPTNGVGYQPYRVVVLSFELLHAPATVCGPKKST

SEQ ID NO: 24 - protein, 204 aa, SARS-CoV-2 Omicron
RFPNITNLCPFDEVFNATRFASVYAWNRKRISNCVADYSVLYNLAPFFTFKCYGVSPTKLNDLCFTNVYADSFVIRGDEVRQIAPGQTGNIADYNYKLPDDFTGCVIAWNSNKLDSKVSGNYNYLYRLFRKSNLKPFERDISTEIYQAGNKPCNGVAGFNCYFPLRSYSFRPTYGVGHQPYRVVVLSFELLHAPATVCGPKKST

SEQ ID NO: 25 - DNA, 26 bp, synthetic construct
  source 1..26: mol_type = other DNA
acaggtacgttaatagttaatagcgt

SEQ ID NO: 26 - DNA, 22 bp, synthetic construct
  source 1..22: mol_type = other DNA
atattgcagcagtacgcacaca

SEQ ID NO: 27 - DNA, 26 bp, synthetic construct
  source 1..26: mol_type = other DNA
acactagccatccttactgcgcttcg

SEQ ID NO: 28 - DNA, 18 bp, synthetic construct
  source 1..18: mol_type = other DNA
atgagcttagtcctgttg

SEQ ID NO: 29 - DNA, 18 bp, synthetic construct
  source 1..18: mol_type = other DNA
ctccctttgttgtgttgt

SEQ ID NO: 30 - DNA, 21 bp, synthetic construct
  source 1..21: mol_type = other DNA
agatgtcttgtgctgccggta

SEQ ID NO: 31 - DNA, 26 bp, synthetic construct
  source 1..26: mol_type = other DNA
acactagccatccttactgcgcttcg

SEQ ID NO: 32 - DNA, 23 bp, synthetic construct
  source 1..23: mol_type = other DNA
cgatctcttgtagatctgttctc

SEQ ID NO: 33 - DNA, 22 bp, synthetic construct
  source 1..22: mol_type = other DNA
atattgcagcagtacgcacaca

SEQ ID NO: 34 - protein, 1251 aa, SARS-CoV-2 Beta
MFVFLVLLPLVSSQCVNFTTRTQLPPAYTNSFTRGVYYPDKVFRSSVLHSTQDLFLPFFSNVTWFHAIHVSGTNGTKRFANPVLPFNDGVYFASTEKSNIIRGWIFGTTLDSKTQSLLIVNNATNVVIKVCEFQFCNDPFLGVYYHKNNKSWMESEFRVYSSANNCTFEYVSQPFLMDLEGKQGNFKNLREFVFKNIDGYFKIYSKHTPINLVRGLPQGFSALEPLVDLPIGINITRFQTLHISYLTPGDSSSGWTAGAAAYYVGYLQPRTFLLKYNENGTITDAVDCALDPLSETKCTLKSFTVEKGIYQTSNFRVQPTESIVRFPNITNLCPFGEVFNATRFASVYAWNRKRISNCVADYSVLYNSASFSTFKCYGVSPTKLNDLCFTNVYADSFVIRGDEVRQIAPGQTGNIADYNYKLPDDFTGCVIAWNSNNLDSKVGGNYNYLYRLFRKSNLKPFERDISTEIYQAGSTPCNGVKGFNCYFPLQSYGFQPTYGVGYQPYRVVVLSFELLHAPATVCGPKKSTNLVKNKCVNFNFNGLTGTGVLTESNKKFLPFQQFGRDIADTTDAVRDPQTLEILDITPCSFGGVSVITPGTNTSNQVAVLYQGVNCTEVPVAIHADQLTPTWRVYSTGSNVFQTRAGCLIGAEHVNNSYECDIPIGAGICASYQTQTNSPRRARSVASQSIIAYTMSLGVENSVAYSNNSIAIPTNFTISVTTEILPVSMTKTSVDCTMYICGDSTECSNLLLQYGSFCTQLNRALTGIAVEQDKNTQEVFAQVKQIYKTPPIKDFGGFNFSQILPDPSKPSKRSFIEDLLFNKVTLADAGFIKQYGDCLGDIAARDLICAQKFNGLTVLPPLLTDEMIAQYTSALLAGTITSGWTFGAGAALQIPFAMQMAYRFNGIGVTQNVLYENQKLIANQFNSAIGKIQDSLSSTASALGKLQDVVNQNAQALNTLVKQLSSNFGAISSVLNDILSRLDKVEAEVQIDRLITGRLQSLQTYVTQQLIRAAEIRASANLAATKMSECVLGQSKRVDFCGKGYHLMSFPQSAPHGVVFLHVTYVPAQEKNFTTAPAICHDGKAHFPREGVFVSNGTHWFVTQRNFYEPQIITTDNTFVSGNCDVVIGIVNNTVYDPLQPELDSFKEELDKYFKNHTSPDVDLGDISGINASVVNIQKEIDRLNEVAKNLNESLIDLQELGKYEQYIKWPWYIWLGFIAGLIAIVMVTIMLCCMTSCCSCLKGCCSCGSCC

SEQ ID NO: 35 - protein, 1252 aa, SARS-CoV-2 Delta
MFVFLVLLPLVSSQCVNLRTRTQLPPAYTNSFTRGVYYPDKVFRSSVLHSTQDLFLPFFSNVTWFHAIHVSGTNGTKRFDNPVLPFNDGVYFASTEKSNIIRGWIFGTTLDSKTQSLLIVNNATNVVIKVCEFQFCNDPFLDVYYHKNNKSWMESGVYSSANNCTFEYVSQPFLMDLEGKQGNFKNLREFVFKNIDGYFKIYSKHTPINLVRDLPQGFSALEPLVDLPIGINITRFQTLLALHRSYLTPGDSSSGWTAGAAAYYVGYLQPRTFLLKYNENGTITDAVDCALDPLSETKCTLKSFTVEKGIYQTSNFRVQPTESIVRFPNITNLCPFGEVFNATRFASVYAWNRKRISNCVADYSVLYNSASFSTFKCYGVSPTKLNDLCFTNVYADSFVIRGDEVRQIAPGQTGKIADYNYKLPDDFTGCVIAWNSNNLDSKVGGNYNYRYRLFRKSNLKPFERDISTEIYQAGSKPCNGVEGFNCYFPLQSYGFQPTNGVGYQPYRVVVLSFELLHAPATVCGPKKSTNLVKNKCVNFNFNGLTGTGVLTESNKKFLPFQQFGRDIADTTDAVRDPQTLEILDITPCSFGGVSVITPGTNTSNQVAVLYQGVNCTEVPVAIHADQLTPTWRVYSTGSNVFQTRAGCLIGAEHVNNSYECDIPIGAGICASYQTQTNSRRRARSVASQSIIAYTMSLGAENSVAYSNNSIAIPTNFTISVTTEILPVSMTKTSVDCTMYICGDSTECSNLLLQYGSFCTQLNRALTGIAVEQDKNTQEVFAQVKQIYKTPPIKDFGGFNFSQILPDPSKPSKRSFIEDLLFNKVTLADAGFIKQYGDCLGDIAARDLICAQKFNGLTVLPPLLTDEMIAQYTSALLAGTITSGWTFGAGAALQIPFAMQMAYRFNGIGVTQNVLYENQKLIANQFNSAIGKIQDSLSSTASALGKLQNVVNQNAQALNTLVKQLSSNFGAISSVLNDILSRLDKVEAEVQIDRLITGRLQSLQTYVTQQLIRAAEIRASANLAATKMSECVLGQSKRVDFCGKGYHLMSFPQSAPHGVVFLHVTYVPAQEKNFTTAPAICHDGKAHFPREGVFVSNGTHWFVTQRNFYEPQIITTDNTFVSGNCDVVIGIVNNTVYDPLQPELDSFKEELDKYFKNHTSPDVDLGDISGINASVVNIQKEIDRLNEVAKNLNESLIDLQELGKYEQYIKWPWYIWLGFIAGLIAIVMVTIMLCCMTSCCSCLKGCCSCGSCC

SEQ ID NO: 36 - protein, 1250 aa, SARS-CoV-2 Omicron
MFVFLVLLPLVSSQCVNLTTRTQLPPAYTNSFTRGVYYPDKVFRSSVLHSTQDLFLPFFSNVTWFHVISGTNGTKRFDNPVLPFNDGVYFASIEKSNIIRGWIFGTTLDSKTQSLLIVNNATNVVIKVCEFQFCNDPFLDHKNNKSWMESEFRVYSSANNCTFEYVSQPFLMDLEGKQGNFKNLREFVFKNIDGYFKIYSKHTPIIVEPEDLPQGFSALEPLVDLPIGINITRFQTLLALHRSYLTPGDSSSGWTAGAAAYYVGYLQPRTFLLKYNENGTITDAVDCALDPLSETKCTLKSFTVEKGIYQTSNFRVQPTESIVRFPNITNLCPFDEVFNATRFASVYAWNRKRISNCVADYSVLYNLAPFFTFKCYGVSPTKLNDLCFTNVYADSFVIRGDEVRQIAPGQTGNIADYNYKLPDDFTGCVIAWNSNKLDSKVSGNYNYLYRLFRKSNLKPFERDISTEIYQAGNKPCNGVAGFNCYFPLRSYSFRPTYGVGHQPYRVVVLSFELLHAPATVCGPKKSTNLVKNKCVNFNFNGLKGTGVLTESNKKFLPFQQFGRDIADTTDAVRDPQTLEILDITPCSFGGVSVITPGTNTSNQVAVLYQGVNCTEVPVAIHADQLTPTWRVYSTGSNVFQTRAGCLIGAEYVNNSYECDIPIGAGICASYQTQTKSHRRARSVASQSIIAYTMSLGAENSVAYSNNSIAIPTNFTISVTTEILPVSMTKTSVDCTMYICGDSTECSNLLLQYGSFCTQLKRALTGIAVEQDKNTQEVFAQVKQIYKTPPIKYFGGFNFSQILPDPSKPSKRSFIEDLLFNKVTLADAGFIKQYGDCLGDIAARDLICAQKFKGLTVLPPLLTDEMIAQYTSALLAGTITSGWTFGAGAALQIPFAMQMAYRFNGIGVTQNVLYENQKLIANQFNSAIGKIQDSLSSTASALGKLQDVVNHNAQALNTLVKQLSSKFGAISSVLNDIFSRLDKVEAEVQIDRLITGRLQSLQTYVTQQLIRAAEIRASANLAATKMSECVLGQSKRVDFCGKGYHLMSFPQSAPHGVVFLHVTYVPAQEKNFTTAPAICHDGKAHFPREGVFVSNGTHWFVTQRNFYEPQIITTDNTFVSGNCDVVIGIVNNTVYDPLQPELDSFKEELDKYFKNHTSPDVDLGDISGINASVVNIQKEIDRLNEVAKNLNESLIDLQELGKYEQYIKWPWYIWLGFIAGLIAIVMVTIMLCCMTSCCSCLKGCCSCGSCC